European Patent Application EP 4 375 369 A1, published May 29, 2024. Title: Novel acetohydroxy acid synthase small subunit variant and a method for producing L-valine acid using the same. Applicant: CJ CheilJedang Corporation. The sequence listing filed with the application follows.

SEQUENCE LISTING (16 sequences)

SEQ ID NO: 1 - protein, 172 aa, Unknown
  Acetohydroxy acid synthase small subunit
MANSDVTRHILSVLVQDVDGIISRVSGMFTRRAFNLVSLVSAKTETLGINRITVVVDADELNIEQITKQLNKLIPVLKVVRLDEETTIARAIMLVKVSADSTNRPQIVDAANIFRARVVDVAPDSVVIESTGTPGKLRALLDVMEPFGIRELIQSGQIALNRGPKTMAPAKI

SEQ ID NO: 2 - DNA, 519 bp, Unknown
  Acetohydroxy acid synthase small subunit
atggctaattctgacgtcacccgccacatcctgtccgtactcgttcaggacgtagacggaatcatttcccgcgtatcaggtatgttcacccgacgcgcattcaacctcgtgtccctcgtgtctgcaaagaccgaaacactcggcatcaaccgcatcacggttgttgtcgacgccgacgagctcaacattgagcagatcaccaagcagctcaacaagctgatccccgtgctcaaagtcgtgcgacttgatgaagagaccaccatcgcccgcgcaatcatgctggttaaggtctctgcggatagcaccaaccgtccgcagatcgtcgacgccgcgaacatcttccgcgcccgagtcgtcgacgtggctccagactctgtggttattgaatccacaggcaccccaggcaagctccgcgcactgcttgatgtgatggaaccattcggaatccgcgaactgatccaatccggacagattgcactcaaccgcggtccgaagaccatggctccggccaagatctaa

SEQ ID NO: 3 - protein, 172 aa, Unknown
  acetohydroxy acid synthase small subunit variant (T44A)
MANSDVTRHILSVLVQDVDGIISRVSGMFTRRAFNLVSLVSAKAETLGINRITVVVDADELNIEQITKQLNKLIPVLKVVRLDEETTIARAIMLVKVSADSTNRPQIVDAANIFRARVVDVAPDSVVIESTGTPGKLRALLDVMEPFGIRELIQSGQIALNRGPKTMAPAKI

SEQ ID NO: 4 - DNA, 519 bp, Unknown
  acetohydroxy acid synthase small subunit variant (T44A)
atggctaattctgacgtcacccgccacatcctgtccgtactcgttcaggacgtagacggaatcatttcccgcgtatcaggtatgttcacccgacgcgcattcaacctcgtgtccctcgtgtctgcaaaggccgaaacactcggcatcaaccgcatcacggttgttgtcgacgccgacgagctcaacattgagcagatcaccaagcagctcaacaagctgatccccgtgctcaaagtcgtgcgacttgatgaagagaccaccatcgcccgcgcaatcatgctggttaaggtctctgcggatagcaccaaccgtccgcagatcgtcgacgccgcgaacatcttccgcgcccgagtcgtcgacgtggctccagactctgtggttattgaatccacaggcaccccaggcaagctccgcgcactgcttgatgtgatggaaccattcggaatccgcgaactgatccaatccggacagattgcactcaaccgcggtccgaagaccatggctccggccaagatctaa

SEQ ID NO: 5 - protein, 172 aa, Unknown
  acetohydroxy acid synthase small subunit variant (T44A+A42V)
MANSDVTRHILSVLVQDVDGIISRVSGMFTRRAFNLVSLVSVKAETLGINRITVVVDADELNIEQITKQLNKLIPVLKVVRLDEETTIARAIMLVKVSADSTNRPQIVDAANIFRARVVDVAPDSVVIESTGTPGKLRALLDVMEPFGIRELIQSGQIALNRGPKTMAPAKI

SEQ ID NO: 6 - DNA, 519 bp, Unknown
  acetohydroxy acid synthase small subunit variant (T44A+A42V)
atggctaattctgacgtcacccgccacatcctgtccgtactcgttcaggacgtagacggaatcatttcccgcgtatcaggtatgttcacccgacgcgcattcaacctcgtgtccctcgtgtctgtaaaggccgaaacactcggcatcaaccgcatcacggttgttgtcgacgccgacgagctcaacattgagcagatcaccaagcagctcaacaagctgatccccgtgctcaaagtcgtgcgacttgatgaagagaccaccatcgcccgcgcaatcatgctggttaaggtctctgcggatagcaccaaccgtccgcagatcgtcgacgccgcgaacatcttccgcgcccgagtcgtcgacgtggctccagactctgtggttattgaatccacaggcaccccaggcaagctccgcgcactgcttgatgtgatggaaccattcggaatccgcgaactgatccaatccggacagattgcactcaaccgcggtccgaagaccatggctccggccaagatctaa

SEQ ID NO: 7 - DNA, 41 bp, Artificial Sequence
  primer
cggggatcctctagaaggacggtactcaaatactaaacttc

SEQ ID NO: 8 - DNA, 41 bp, Artificial Sequence
  primer
cggggatcctctagagacaactacattattattataccaca

SEQ ID NO: 9 - DNA, 41 bp, Artificial Sequence; identical to SEQ ID NO: 7
  primer

SEQ ID NO: 10 - DNA, 28 bp, Artificial Sequence
  primer
ggcctttgcagacacgagggacacgagg

SEQ ID NO: 11 - DNA, 35 bp, Artificial Sequence
  primer
tgtccctcgtgtctgcaaaggccgaaacactcggc

SEQ ID NO: 12 - DNA, 41 bp, Artificial Sequence; identical to SEQ ID NO: 8
  primer

SEQ ID NO: 13 - DNA, 41 bp, Artificial Sequence; identical to SEQ ID NO: 7
  primer

SEQ ID NO: 14 - DNA, 38 bp, Artificial Sequence
  primer
tgccgagtgtttcggtctttacagacacgagggacacg

SEQ ID NO: 15 - DNA, 31 bp, Artificial Sequence
  primer odhA_down_F
tgtctgtaaagaccgaaacactcggcatcaa

SEQ ID NO: 16 - DNA, 41 bp, Artificial Sequence; identical to SEQ ID NO: 8
  primer